European Patent Specification EP 3 717 007 B1, published September 17, 2025. Title: ILDR2 antagonists, and combinations thereof. Applicant: Bayer Intellectual Property GmbH. The sequence listing filed with the application follows.

SEQUENCE LISTING (51 sequences)

SEQ ID NO: 1 - protein, 5 aa, artificial
  59-08.B02 BAY1905254 HCDR1
SYAIS

SEQ ID NO: 2 - protein, 17 aa, artificial
  59-08.B02 BAY1905254 HCDR2
GIIPILGIANYAQKFQG

SEQ ID NO: 3 - protein, 13 aa, Artificial
  59-08.B02 BAY1905254 HCDR3
ARGRLPYGDFWDS

SEQ ID NO: 4 - protein, 16 aa, Artificial
  59-08.B02 BAY1905254 LCDR1
RSSQSLLYSNGYNYLD

SEQ ID NO: 5 - protein, 7 aa, Artificial
  59-08.B02 BAY1905254 LCDR2
LGSNRAS

SEQ ID NO: 6 - protein, 9 aa, Artificial
  59-08.B02 BAY1905254 LCDR3
MQALQTPLT

SEQ ID NO: 7 - protein, 120 aa, Artificial
  59-08.B02 heavy chain VD| BAY1905254
QVQLVQSGAEVKKPGSSVKVSCKASGGTFSSYAISWVRQAPGQGLEWMGGIIPILGIANYAQKFQGRVTITADKSTSTAYMELSSLRSEDTAVYYCARGRLPYGDFWDSWGQGTLVTVSS

SEQ ID NO: 8 - protein, 112 aa, Artificial
  59-08.B02-light chain VD| BAY1905254
DIVMTQSPLSLPVTPGEPASISCRSSQSLLYSNGYNYLDWYLQKPGQSPQLLIYLGSNRASGVPDRFSGSGSGTDFTLKISRVEAEDVGVYYCMQALQTPLTFGGGTKLEIR

SEQ ID NO: 9 - protein, 121 aa, Artificial
  61-02.C05 heavy chain VD
EVQLVESGGGVVQPGGSLRLSCAASGFTFSSYAMSWVRQAPGKGLEWVSGISSSGGSTQYADSVKGRFTVSRDNSKNTLYLQMKSLRAEDTALYYCAKDFVGVLPDAFDIWGQGTMVTVSS

SEQ ID NO: 10 - protein, 107 aa, Artificial
  61-02.C05 light chain VD
DIQLTQSPSSLSASVGDRVTITCQASQDTNKYLNWYQQKPGKAPELLIYGASTLESGVPPRFSASGSGTDFTLTINSLQPEDIGRYYCQQYHIPPPSFGGGTKLEIK

SEQ ID NO: 11 - protein, 115 aa, Artificial
  56-02.E08 heavy chain VD
EVQLVQSGAEVKKPGESLKISCKASGYSFTTYWIGWVRQVPGKGLEWMGIIYPGDYDTRYSPSFQGQVTISADKSINTAYLQWSSLEASDSAMYYCAIGEPFDYWGQGTLVTVSS

SEQ ID NO: 12 - protein, 112 aa, Artificial
  56-02.E08 light chain VD
DVVMTQSPLSLPVTPGEPASISCRSSQSLLHANGYNYLDWYLQKPGQSPQLLIYLGSNRASGVPDRFSGSGSGTDFTLKISRVETEDVGVYYCMQALQTPLTFGGGTKVEIK

SEQ ID NO: 13 - protein, 131 aa, artificial
  74.15.G09 heavy chain VD
EVQLVESGGGVVQPGRSLRLSCAASGFTFSSYGMHWVRQAPGKGLEWVAVISYDGSNKYYADSVKGRFTISRDNSKNTLYLQMNSLRAEDTAVYYCAKESPSVGLGSYYDFWSGLYGMDVWGQGTTVTVSS

SEQ ID NO: 14 - protein, 108 aa, Artificial
  74.15.G09 light chain VD
EIVLTQSPGTLSLSPGERVTLSCRTGQRVENLFIAWYQQKPGQAPRLLLYGASNRATGIPDRFSGSGSGTDFTLTISRLEPEDSAVYYCQQYDDSGITFGQGTRLEIK

SEQ ID NO: 15 - protein, 125 aa, Artificial
  56.02.E10 heavy chain VD
QVQLVESGGGLVKPGGSLRLSCAASGFTFSNYGMHWVRQAPGKGPEWLAFIRYDGSKKYYADSVRGRFTISRDNSKNMLYLQMNSLRTEDTAVYYCAKEGIAAPGSGYYYGMDVWGQGTTVTVSS

SEQ ID NO: 16 - protein, 109 aa, Artificial
  56.02.E10 light chain VD
QSALTQPASVSGSPGQSITISCSGTTTDVGRYTLVSWYQHHPGKAPKLIIFEVNKRPSGVSSRFSGSKSGNTASLTISGLQTEDEADYFCCSYTGTTVIFGGGTQLTVL

SEQ ID NO: 17 - DNA, 20 bp, Artificial
  CPG Oligo nucleotide ODN 1826
tccatgacgttcctgacgtt

SEQ ID NO: 18 - protein, 5 aa, Artificial
  61-02.C05 HCDR1
SYAMS

SEQ ID NO: 19 - protein, 17 aa, Artificial
  61-02.C05 HCDR2
GISSSGGSTQYADSVKG

SEQ ID NO: 20 - protein, 12 aa, Artificial
  61-02.C05 HCDR3
DFVGVLPDAFDI

SEQ ID NO: 21 - protein, 11 aa, artificial
  61-02.C05 LCDR1
QASQDTNKYLN

SEQ ID NO: 22 - protein, 7 aa, Artificial
  61-02.C05 LCDR2
GASTLES

SEQ ID NO: 23 - protein, 9 aa, Artificial
  61-02.C05 LCDR3
QQYHIPPPS

SEQ ID NO: 24 - protein, 5 aa, Artificial
  56-02.E08 HCDR1
TYWIG

SEQ ID NO: 25 - protein, 17 aa, Artificial
  56-02.E08 HCDR2
IIYPGDYDTRYSPSFQG

SEQ ID NO: 26 - protein, 8 aa, Artificial
  56-02.E08 HCDR3
AIGEPFDY

SEQ ID NO: 27 - protein, 16 aa, Artificial
  56-02.E08 LCDR1
RSSQSLLHANGYNYLD

SEQ ID NO: 28 - protein, 7 aa, Artificial
  56-02.E08 LCDR2
LGSNRAS

SEQ ID NO: 29 - protein, 9 aa, Artificial
  56-02.E08 LCDR3
MQALQTPLT

SEQ ID NO: 30 - protein, 5 aa, Artificial
  74.15.G09 HCDR1
SYGMH

SEQ ID NO: 31 - protein, 17 aa, Artificial
  74.15.G09 HCDR2
VISYDGSNKYYADSVKG

SEQ ID NO: 32 - protein, 24 aa, Artificial
  74.15.G09 HCDR3
AKESPSVGLGSYYDFWSGLYGMDV

SEQ ID NO: 33 - protein, 12 aa, Artificial
  74.15.G09 LCDR1
RTGQRVENLFIA

SEQ ID NO: 34 - protein, 7 aa, Artificial
  74.15.G09 LCDR2
GASNRAT

SEQ ID NO: 35 - protein, 9 aa, Artificial
  74.15.G09 LCDR3
QQYDDSGIT

SEQ ID NO: 36 - protein, 5 aa, Artificial
  56.02.E10 HCDR1
NYGMH

SEQ ID NO: 37 - protein, 17 aa, Artificial
  56.02.E10 HCDR2
FIRYDGSKKYYADSVRG

SEQ ID NO: 38 - protein, 16 aa, Artificial
  56.02.E10 HCDR3
EGIAAPGSGYYYGMDV

SEQ ID NO: 39 - protein, 14 aa, Artificial
  56.02.E10 LCDR1
SGTTTDVGRYTLVS

SEQ ID NO: 40 - protein, 7 aa, Artificial
  56.02.E10 LCDR2
EVNKRPS

SEQ ID NO: 41 - protein, 9 aa, Artificial
  56.02.E10 LCDR3
CSYTGTTVI

SEQ ID NO: 42 - protein, 445 aa, Artificial
  59-08.B02 heavy chain BAY1905254
QVQLVQSGAEVKKPGSSVKVSCKASGGTFSSYAISWVRQAPGQGLEWMGGIIPILGIANYAQKFQGRVTITADKSTSTAYMELSSLRSEDTAVYYCARGRLPYGDFWDSWGQGTLVTVSSASTKGPSVFPLAPCSRSTSESTAALGCLVKDYFPEPVTVSWNSGALTSGVHTFPAVLQSSGLYSLSSVVTVPSSNFGTQTYTCNVDHKPSNTKVDKTVERKCCVECPPCPAPPVAGPSVFLFPPKPKDTLMISRTPEVTCVVVDVSHEDPEVQFNWYVDGVEVHNAKTKPREEQFNSTFRVVSVLTVVHQDWLNGKEYKCKVSNKGLPAPIEKTISKTKGQPREPQVYTLPPSREEMTKNQVSLTCLVKGFYPSDIAVEWESNGQPENNYKTTPPMLDSDGSFFLYSKLTVDKSRWQQGNVFSCSVMHEALHNHYTQKSLSLSPG

SEQ ID NO: 43 - protein, 219 aa, Artificial
  59-08.B02-light chain BAY1905254
DIVMTQSPLSLPVTPGEPASISCRSSQSLLYSNGYNYLDWYLQKPGQSPQLLIYLGSNRASGVPDRFSGSGSGTDFTLKISRVEAEDVGVYYCMQALQTPLTFGGGTKLEIRRTVAAPSVFIFPPSDEQLKSGTASVVCLLNNFYPREAKVQWKVDNALQSGNSQESVTEQDSKDSTYSLSSTLTLSKADYEKHKVYACEVTHQGLSSPVTKSFNRGEC

SEQ ID NO: 44 - protein, 446 aa, Artificial
  61-02.C05 heavy chain
EVQLVESGGGVVQPGGSLRLSCAASGFTFSSYAMSWVRQAPGKGLEWVSGISSSGGSTQYADSVKGRFTVSRDNSKNTLYLQMKSLRAEDTALYYCAKDFVGVLPDAFDIWGQGTMVTVSSASTKGPSVFPLAPCSRSTSESTAALGCLVKDYFPEPVTVSWNSGALTSGVHTFPAVLQSSGLYSLSSVVTVPSSNFGTQTYTCNVDHKPSNTKVDKTVERKCCVECPPCPAPPVAGPSVFLFPPKPKDTLMISRTPEVTCVVVDVSHEDPEVQFNWYVDGVEVHNAKTKPREEQFNSTFRVVSVLTVVHQDWLNGKEYKCKVSNKGLPAPIEKTISKTKGQPREPQVYTLPPSREEMTKNQVSLTCLVKGFYPSDIAVEWESNGQPENNYKTTPPMLDSDGSFFLYSKLTVDKSRWQQGNVFSCSVMHEALHNHYTQKSLSLSPG

SEQ ID NO: 45 - protein, 214 aa, Artificial
  61-02.C05 light chain
DIQLTQSPSSLSASVGDRVTITCQASQDTNKYLNWYQQKPGKAPELLIYGASTLESGVPPRFSASGSGTDFTLTINSLQPEDIGRYYCQQYHIPPPSFGGGTKLEIKRTVAAPSVFIFPPSDEQLKSGTASVVCLLNNFYPREAKVQWKVDNALQSGNSQESVTEQDSKDSTYSLSSTLTLSKADYEKHKVYACEVTHQGLSSPVTKSFNRGEC

SEQ ID NO: 46 - protein, 440 aa, Artificial
  56-02.E08 heavy chain
EVQLVQSGAEVKKPGESLKISCKASGYSFTTYWIGWVRQVPGKGLEWMGIIYPGDYDTRYSPSFQGQVTISADKSINTAYLQWSSLEASDSAMYYCAIGEPFDYWGQGTLVTVSSASTKGPSVFPLAPCSRSTSESTAALGCLVKDYFPEPVTVSWNSGALTSGVHTFPAVLQSSGLYSLSSVVTVPSSNFGTQTYTCNVDHKPSNTKVDKTVERKCCVECPPCPAPPVAGPSVFLFPPKPKDTLMISRTPEVTCVVVDVSHEDPEVQFNWYVDGVEVHNAKTKPREEQFNSTFRVVSVLTVVHQDWLNGKEYKCKVSNKGLPAPIEKTISKTKGQPREPQVYTLPPSREEMTKNQVSLTCLVKGFYPSDIAVEWESNGQPENNYKTTPPMLDSDGSFFLYSKLTVDKSRWQQGNVFSCSVMHEALHNHYTQKSLSLSPG

SEQ ID NO: 47 - protein, 219 aa, Artificial
  56-02.E08 light chain
DVVMTQSPLSLPVTPGEPASISCRSSQSLLHANGYNYLDWYLQKPGQSPQLLIYLGSNRASGVPDRFSGSGSGTDFTLKISRVETEDVGVYYCMQALQTPLTFGGGTKVEIKRTVAAPSVFIFPPSDEQLKSGTASVVCLLNNFYPREAKVQWKVDNALQSGNSQESVTEQDSKDSTYSLSSTLTLSKADYEKHKVYACEVTHQGLSSPVTKSFNRGEC

SEQ ID NO: 48 - protein, 456 aa, Artificial
  74.15.G09 heavy chain
EVQLVESGGGVVQPGRSLRLSCAASGFTFSSYGMHWVRQAPGKGLEWVAVISYDGSNKYYADSVKGRFTISRDNSKNTLYLQMNSLRAEDTAVYYCAKESPSVGLGSYYDFWSGLYGMDVWGQGTTVTVSSASTKGPSVFPLAPCSRSTSESTAALGCLVKDYFPEPVTVSWNSGALTSGVHTFPAVLQSSGLYSLSSVVTVPSSNFGTQTYTCNVDHKPSNTKVDKTVERKCCVECPPCPAPPVAGPSVFLFPPKPKDTLMISRTPEVTCVVVDVSHEDPEVQFNWYVDGVEVHNAKTKPREEQFNSTFRVVSVLTVVHQDWLNGKEYKCKVSNKGLPAPIEKTISKTKGQPREPQVYTLPPSREEMTKNQVSLTCLVKGFYPSDIAVEWESNGQPENNYKTTPPMLDSDGSFFLYSKLTVDKSRWQQGNVFSCSVMHEALHNHYTQKSLSLSPG

SEQ ID NO: 49 - protein, 215 aa, Artificial
  74.15.G09 light chain
EIVLTQSPGTLSLSPGERVTLSCRTGQRVENLFIAWYQQKPGQAPRLLLYGASNRATGIPDRFSGSGSGTDFTLTISRLEPEDSAVYYCQQYDDSGITFGQGTRLEIKRTVAAPSVFIFPPSDEQLKSGTASVVCLLNNFYPREAKVQWKVDNALQSGNSQESVTEQDSKDSTYSLSSTLTLSKADYEKHKVYACEVTHQGLSSPVTKSFNRGEC

SEQ ID NO: 50 - protein, 450 aa, Artificial
  56.02.E10 heavy chain
QVQLVESGGGLVKPGGSLRLSCAASGFTFSNYGMHWVRQAPGKGPEWLAFIRYDGSKKYYADSVRGRFTISRDNSKNMLYLQMNSLRTEDTAVYYCAKEGIAAPGSGYYYGMDVWGQGTTVTVSSASTKGPSVFPLAPCSRSTSESTAALGCLVKDYFPEPVTVSWNSGALTSGVHTFPAVLQSSGLYSLSSVVTVPSSNFGTQTYTCNVDHKPSNTKVDKTVERKCCVECPPCPAPPVAGPSVFLFPPKPKDTLMISRTPEVTCVVVDVSHEDPEVQFNWYVDGVEVHNAKTKPREEQFNSTFRVVSVLTVVHQDWLNGKEYKCKVSNKGLPAPIEKTISKTKGQPREPQVYTLPPSREEMTKNQVSLTCLVKGFYPSDIAVEWESNGQPENNYKTTPPMLDSDGSFFLYSKLTVDKSRWQQGNVFSCSVMHEALHNHYTQKSLSLSPG

SEQ ID NO: 51 - protein, 215 aa, Artificial
  56.02.E10 light chain
QSALTQPASVSGSPGQSITISCSGTTTDVGRYTLVSWYQHHPGKAPKLIIFEVNKRPSGVSSRFSGSKSGNTASLTISGLQTEDEADYFCCSYTGTTVIFGGGTQLTVLGQPKAAPSVTLFPPSSEELQANKATLVCLISDFYPGAVTVAWKADSSPVKAGVETTTPSKQSNNKYAASSYLSLTPEQWKSHRSYSCQVTHEGSTVEKTVAPTECS